European Patent Application EP 4 643 894 A1, published November 5, 2025. Title: Method for producing retinal sheet. Applicant: VCCT Inc. The sequence listing filed with the application follows.

SEQUENCE LISTING (90 sequences)

SEQ ID NO: 1 - DNA, 19 bp, synthetic construct
  source 1..19: mol_type = other DNA
acatcgctcagacaccatg

SEQ ID NO: 2 - DNA, 22 bp, synthetic construct
  source 1..22: mol_type = other DNA
tgtagttgaggtcaatgaaggg

SEQ ID NO: 3 - DNA, 20 bp, synthetic construct
  source 1..20: mol_type = other DNA
cgacctggaagtccaactac

SEQ ID NO: 4 - DNA, 18 bp, synthetic construct
  source 1..18: mol_type = other DNA
atctgctgcatctgcttg

SEQ ID NO: 5 - DNA, 20 bp, synthetic construct
  source 1..20: mol_type = other DNA
ccccactattctgtcaacgc

SEQ ID NO: 6 - DNA, 18 bp, synthetic construct
  source 1..18: mol_type = other DNA
aaacagtgcctccagctc

SEQ ID NO: 7 - DNA, 20 bp, synthetic construct
  source 1..20: mol_type = other DNA
tgcgggctactgaaaagttc

SEQ ID NO: 8 - DNA, 19 bp, synthetic construct
  source 1..19: mol_type = other DNA
ggctgagggacatcttgag

SEQ ID NO: 9 - DNA, 17 bp, synthetic construct
  source 1..17: mol_type = other DNA
aggagacaggagcccag

SEQ ID NO: 10 - DNA, 19 bp, synthetic construct
  source 1..19: mol_type = other DNA
gcacagacatcgagaccag

SEQ ID NO: 11 - DNA, 19 bp, synthetic construct
  source 1..19: mol_type = other DNA
taacgggaccatcagcaag

SEQ ID NO: 12 - DNA, 21 bp, synthetic construct
  source 1..21: mol_type = other DNA
tcctcgggagtgatcattttg

SEQ ID NO: 13 - DNA, 18 bp, synthetic construct
  source 1..18: mol_type = other DNA
caaccccagcaagaaacg

SEQ ID NO: 14 - DNA, 17 bp, synthetic construct
  source 1..17: mol_type = other DNA
ctcggtccaatggcctg

SEQ ID NO: 15 - DNA, 17 bp, synthetic construct
  source 1..17: mol_type = other DNA
gacaaagggaccgagcg

SEQ ID NO: 16 - DNA, 19 bp, synthetic construct
  source 1..19: mol_type = other DNA
cttgctggatagactggcg

SEQ ID NO: 17 - DNA, 20 bp, synthetic construct
  source 1..20: mol_type = other DNA
accagaccaagaaacggaag

SEQ ID NO: 18 - DNA, 20 bp, synthetic construct
  source 1..20: mol_type = other DNA
ttgaatgccttctccagctc

SEQ ID NO: 19 - DNA, 19 bp, synthetic construct
  source 1..19: mol_type = other DNA
cctacacgcatcccagttc

SEQ ID NO: 20 - DNA, 18 bp, synthetic construct
  source 1..18: mol_type = other DNA
ttgtggtcgggttgtctg

SEQ ID NO: 21 - DNA, 19 bp, synthetic construct
  source 1..19: mol_type = other DNA
cttccgtgccctcatgtac

SEQ ID NO: 22 - DNA, 19 bp, synthetic construct
  source 1..19: mol_type = other DNA
agttcacaccatcagccag

SEQ ID NO: 23 - DNA, 20 bp, synthetic construct
  source 1..20: mol_type = other DNA
tggaacacgcctttgagaag

SEQ ID NO: 24 - DNA, 20 bp, synthetic construct
  source 1..20: mol_type = other DNA
ccagcttctgccttttgaac

SEQ ID NO: 25 - DNA, 18 bp, synthetic construct
  source 1..18: mol_type = other DNA
agaaacccagccaatccg

SEQ ID NO: 26 - DNA, 18 bp, synthetic construct
  source 1..18: mol_type = other DNA
tgttggtgtaagccgtgc

SEQ ID NO: 27 - DNA, 20 bp, synthetic construct
  source 1..20: mol_type = other DNA
cgttcgagaagtcccactac

SEQ ID NO: 28 - DNA, 20 bp, synthetic construct
  source 1..20: mol_type = other DNA
gacacttccagcttctcctg

SEQ ID NO: 29 - DNA, 21 bp, synthetic construct
  source 1..21: mol_type = other DNA
tcactcgccacatctactttg

SEQ ID NO: 30 - DNA, 20 bp, synthetic construct
  source 1..20: mol_type = other DNA
caggttcagagtccttggtg

SEQ ID NO: 31 - DNA, 20 bp, synthetic construct
  source 1..20: mol_type = other DNA
cacccagctctcagctaaat

SEQ ID NO: 32 - DNA, 21 bp, synthetic construct
  source 1..21: mol_type = other DNA
ggtggatgggtagttcatgtt

SEQ ID NO: 33 - DNA, 22 bp, synthetic construct
  source 1..22: mol_type = other DNA
cctgatcagagagcaggaaatg

SEQ ID NO: 34 - DNA, 21 bp, synthetic construct
  source 1..21: mol_type = other DNA
ccttccggttgtaaggagttt

SEQ ID NO: 35 - DNA, 21 bp, synthetic construct
  source 1..21: mol_type = other DNA
gcggaagctgcaaagaaatag

SEQ ID NO: 36 - DNA, 22 bp, synthetic construct
  source 1..22: mol_type = other DNA
gggcaaacacatctggataatg

SEQ ID NO: 37 - DNA, 22 bp, synthetic construct
  source 1..22: mol_type = other DNA
ggagagtaagaaacagcatgga

SEQ ID NO: 38 - DNA, 20 bp, synthetic construct
  source 1..20: mol_type = other DNA
gtggatgggattggtgttct

SEQ ID NO: 39 - DNA, 20 bp, synthetic construct
  source 1..20: mol_type = other DNA
ccaggccgaagttccattta

SEQ ID NO: 40 - DNA, 23 bp, synthetic construct
  source 1..23: mol_type = other DNA
ccacccagaagtaaccactattc

SEQ ID NO: 41 - DNA, 23 bp, synthetic construct
  source 1..23: mol_type = other DNA
gtcctctcaacttccagatacac

SEQ ID NO: 42 - DNA, 20 bp, synthetic construct
  source 1..20: mol_type = other DNA
ttcccactttctccaacagg

SEQ ID NO: 43 - DNA, 23 bp, synthetic construct
  source 1..23: mol_type = other DNA
cggcttaaattggactcctagat

SEQ ID NO: 44 - DNA, 21 bp, synthetic construct
  source 1..21: mol_type = other DNA
gctgtggctaagtgggaaata

SEQ ID NO: 45 - DNA, 21 bp, synthetic construct
  source 1..21: mol_type = other DNA
aaccagaggcagaaacagaaa

SEQ ID NO: 46 - DNA, 21 bp, synthetic construct
  source 1..21: mol_type = other DNA
aggcagaagagaggagagaaa

SEQ ID NO: 47 - DNA, 21 bp, synthetic construct
  source 1..21: mol_type = other DNA
gcttggctgtttagtggtttg

SEQ ID NO: 48 - DNA, 22 bp, synthetic construct
  source 1..22: mol_type = other DNA
gtggcatggtagaacagatgag

SEQ ID NO: 49 - RNA, 20 nt, synthetic construct
  source 1..20: mol_type = other RNA
cgcctctttgaccagttctt

SEQ ID NO: 50 - DNA, 22 bp, synthetic construct
  source 1..22: mol_type = other DNA
tagaagggactcagggaagtag

SEQ ID NO: 51 - DNA, 20 bp, synthetic construct
  source 1..20: mol_type = other DNA
aagtttcccaccaggatgac

SEQ ID NO: 52 - DNA, 21 bp, synthetic construct
  source 1..21: mol_type = other DNA
caacgctctgaacctctcttt

SEQ ID NO: 53 - DNA, 22 bp, synthetic construct
  source 1..22: mol_type = other DNA
cgcagacggaaatgggtatatt

SEQ ID NO: 54 - DNA, 20 bp, synthetic construct
  source 1..20: mol_type = other DNA
gacatcatgccagagccttt

SEQ ID NO: 55 - DNA, 21 bp, synthetic construct
  source 1..21: mol_type = other DNA
tgtggtattgtcgggactttg

SEQ ID NO: 56 - DNA, 20 bp, synthetic construct
  source 1..20: mol_type = other DNA
tcagtgctcggttgctttag

SEQ ID NO: 57 - DNA, 22 bp, synthetic construct
  source 1..22: mol_type = other DNA
gtccctcctactgtgtgttatg

SEQ ID NO: 58 - DNA, 22 bp, synthetic construct
  source 1..22: mol_type = other DNA
ccctactaatgggatggatgag

SEQ ID NO: 59 - DNA, 20 bp, synthetic construct
  source 1..20: mol_type = other DNA
tcatccccatttccttcgtg

SEQ ID NO: 60 - DNA, 18 bp, synthetic construct
  source 1..18: mol_type = other DNA
ttgctcgtccttgccttc

SEQ ID NO: 61 - DNA, 18 bp, synthetic construct
  source 1..18: mol_type = other DNA
tggcggtcttcagttgtg

SEQ ID NO: 62 - DNA, 21 bp, synthetic construct
  source 1..21: mol_type = other DNA
ggaacccaggagatcagaatg

SEQ ID NO: 63 - DNA, 21 bp, synthetic construct
  source 1..21: mol_type = other DNA
aggaaatcttgggcttgatgg

SEQ ID NO: 64 - DNA, 18 bp, synthetic construct
  source 1..18: mol_type = other DNA
tgttgggaaggttggctg

SEQ ID NO: 65 - DNA, 20 bp, synthetic construct
  source 1..20: mol_type = other DNA
agaacatgtgtaagctgcgg

SEQ ID NO: 66 - DNA, 19 bp, synthetic construct
  source 1..19: mol_type = other DNA
gttgcctctcactcggttc

SEQ ID NO: 67 - DNA, 20 bp, synthetic construct
  source 1..20: mol_type = other DNA
gaaatacctcagcctccagc

SEQ ID NO: 68 - DNA, 20 bp, synthetic construct
  source 1..20: mol_type = other DNA
gcgtcacaccattgctattc

SEQ ID NO: 69 - DNA, 21 bp, synthetic construct
  source 1..21: mol_type = other DNA
gacagtcggttttcccatttg

SEQ ID NO: 70 - DNA, 22 bp, synthetic construct
  source 1..22: mol_type = other DNA
tcccagtttgctgatttcattg

SEQ ID NO: 71 - DNA, 24 bp, synthetic construct
  source 1..24: mol_type = other DNA
gggataaaggctacttaacaaagg

SEQ ID NO: 72 - DNA, 22 bp, synthetic construct
  source 1..22: mol_type = other DNA
ccactttgccatctctacactg

SEQ ID NO: 73 - DNA, 21 bp, synthetic construct
  source 1..21: mol_type = other DNA
catcaaaactgtcaccgaagc

SEQ ID NO: 74 - DNA, 20 bp, synthetic construct
  source 1..20: mol_type = other DNA
tccaagtcaacctttccacc

SEQ ID NO: 75 - DNA, 18 bp, synthetic construct
  source 1..18: mol_type = other DNA
cgctgacccacatctgag

SEQ ID NO: 76 - DNA, 20 bp, synthetic construct
  source 1..20: mol_type = other DNA
tcatcggtacaaggcaacag

SEQ ID NO: 77 - DNA, 20 bp, synthetic construct
  source 1..20: mol_type = other DNA
accaactgagccaacatgtg

SEQ ID NO: 78 - DNA, 22 bp, synthetic construct
  source 1..22: mol_type = other DNA
gagttctcgaaaagccaggtag

SEQ ID NO: 79 - DNA, 21 bp, synthetic construct
  source 1..21: mol_type = other DNA
cactgtggacattactccctc

SEQ ID NO: 80 - DNA, 19 bp, synthetic construct
  source 1..19: mol_type = other DNA
ccgcatgccattccaaatc

SEQ ID NO: 81 - DNA, 19 bp, synthetic construct
  source 1..19: mol_type = other DNA
tcaagctgccagaagatgc

SEQ ID NO: 82 - DNA, 17 bp, synthetic construct
  source 1..17: mol_type = other DNA
tgtgtttgcggagggtg

SEQ ID NO: 83 - DNA, 17 bp, synthetic construct
  source 1..17: mol_type = other DNA
cctgccctgacaagtgc

SEQ ID NO: 84 - DNA, 17 bp, synthetic construct
  source 1..17: mol_type = other DNA
cagtcacaggggcgatc

SEQ ID NO: 85 - DNA, 22 bp, synthetic construct
  source 1..22: mol_type = other DNA
ctggtgtcctacaaagtcagag

SEQ ID NO: 86 - DNA, 20 bp, synthetic construct
  source 1..20: mol_type = other DNA
tcatgagatggcttcggatg

SEQ ID NO: 87 - DNA, 22 bp, synthetic construct
  source 1..22: mol_type = other DNA
ccagaaaaggctcaacatcaac

SEQ ID NO: 88 - DNA, 18 bp, synthetic construct
  source 1..18: mol_type = other DNA
ttccaccgtgtccacatg

SEQ ID NO: 89 - DNA, 18 bp, synthetic construct
  source 1..18: mol_type = other DNA
cagcgactcggtccaatc

SEQ ID NO: 90 - DNA, 20 bp, synthetic construct
  source 1..20: mol_type = other DNA
agacataaggcctcggtagt